European Patent Specification EP 3 628 744 B1, published November 1, 2023. Title: Intracellular recording method using the membrane penetrating nanoparticles as an electrode (nanoelectrode). Applicant: Ion Chat Research Corporation Saito, Mitsuyoshi. The sequence listing filed with the application follows.

SEQUENCE LISTING (6 sequences)

SEQ ID NO: 1 - DNA, 38 bp, Artificial Sequence
  ChRWR sense primer
cactatagggaagctaccatggctcggagaccctggct

SEQ ID NO: 2 - DNA, 38 bp, Artificial Sequence
  ChRWR antisense primer
atagaataggaagctctacttgcctgtccctttgttga

SEQ ID NO: 3 - DNA, 20 bp, Artificial Sequence
  KIR2.1 1st sense primer
ccaaagcagaagcactggag

SEQ ID NO: 4 - DNA, 22 bp, Artificial Sequence
  KIR2.1 1st A/S
ctttgaaaccattgtgcttgcc

SEQ ID NO: 5 - DNA, 39 bp, Artificial Sequence
  KIR2.1 ICR HindIII sense
cactatagggaagctaccatgggcagtgtgcgaaccaac

SEQ ID NO: 6 - DNA, 36 bp, Artificial Sequence
  KIR2.1 ICR HindIII A/S
atagaataggaagcttcatatctccgactctcgccg